European Patent Specification EP 3 559 279 B1, published June 26, 2024. Title: STREPTOCOCCUS THERMOPHILUS STARTER CULTURES. Applicant: DSM IP Assets B.V. The sequence listing filed with the application follows.

SEQUENCE LISTING (17 sequences)

SEQ ID NO: 1 - DNA, 21 bp, Artificial Sequence
  RGP group1 forward primer
ggatgatggttcgacggatag

SEQ ID NO: 2 - DNA, 20 bp, Artificial Sequence
  RGP group1 reverse primer
ccgctcttccaaaaccatga

SEQ ID NO: 3 - DNA, 631 bp, Streptococcus thermophilus
  RGP group1 amplicon
ggatgatggttcgacggatagttcaactcaaattatccaagaggttttgaaggattcaccttttgagacaagatttgaaactcatgaaaaccttggggtagtaaagaatcgaaatttaggattagagcttataagaggtgactatttgctatttgtagatagtgataactacctcgatgcggattatgtggaacagttgtacagtaagttgacggaaacaaatgctgatattgcgtactgtgatctttttaatccagaaaaagaagagttctaccttaaaagccgtgaatttgacctaactgcctttctaaatgctagttttattgataactgttctttgattcgtagaagtattattggaaatgctcgttatgatgagatgttaaatcgtaaaaagcttgaagattatgactttttattgaacttaatcattaataacggtgctaaagcggtatatcaaccaagcactaagcttaattatcgtgtctttgaaacaggatcaatttctggacgtgactccgttcgctaccattatgaaatctatcttgacattcttgagaagtaccttgataagcttcctcatgaaatttacaaggcagtttgtgagaacctcatggttttggaagagcgg

SEQ ID NO: 4 - DNA, 21 bp, Artificial Sequence
  RGP group2 forward primer
gtgaagagtcagaagacgaat

SEQ ID NO: 5 - DNA, 19 bp, Artificial Sequence
  RGP group2 reverse primer
caaaggccccgatggtatt

SEQ ID NO: 6 - DNA, 464 bp, Streptococcus thermophilus
  RGP group2 amplicon
gtgaagagtcagaagacgaataattgatttgtttttatattcatagcaatggcgacttgaacagtcgcttttctttttgtattaggaaaaaagcccagaaaatggtataattgagtggattgtaatttgtaagaaaggaaataatatgcaacacgtttttattatcggaagtcgtggacttccggctcaatatggtggtttcgagaccttcgtggaccaattggtctccaatcgagtatcaccgaatatcaagtaccatgttgcttgcctttctaatgatcaagcctactatcattttgactacaagggtgtagattgttttacgattaaagcacccaaacttgggcctgcgcgggtcattgcctatgatatgatggccatcaattatgccttgaaggtcattaagaaacaaggaattgaaaaacctattttttatattttgggcaataccatcggggcctttg

SEQ ID NO: 7 - DNA, 21 bp, Artificial Sequence
  RGP group3 forward primer
gaggaagcaacagataaacga

SEQ ID NO: 8 - DNA, 21 bp, Artificial Sequence
  RGP group3 reverse primer
gaccaattggtccacaaaagt

SEQ ID NO: 9 - DNA, 303 bp, Streptococcus thermophilus
  RGP group3 amplicon
gaggaagcaacagataaacgagaatattttgtttatgttattgccaatctatttatattgatgtcagtagtattgacaatccttcagtactatggtgtgaaaaataatttttaacttttttcaagtagtcctttgtggctgcttttctgtttgcaataggcaaaatctttgtaaaatggtataattgactagattatagacttgttagaaaggggatttatgcaacaacacgtattcattattggaagtcgtgggcttccgtctcaatatggcggttttgagacttttgtggaccaattggtc

SEQ ID NO: 10 - DNA, 18 bp, Artificial Sequence
  RGP group4 forward primer
ctcctcgtactcacccac

SEQ ID NO: 11 - DNA, 21 bp, Artificial Sequence
  RGP group4 reverse primer
gcacaagatacagctcgttac

SEQ ID NO: 12 - DNA, 162 bp, Streptococcus thermophilus
  RGP group4 amplicon
ctcctcgtactcacccacaattttttcccaagtaaagttctgtttcatattctccttagctaacttacctagttcagagtaatctgaaatagcatctacttggtcaatcaaatgcgacagattgccctcatcttttttccagtaacgagctgtatcttgtgc

SEQ ID NO: 13 - DNA, 21 bp, Artificial Sequence
  RGP group positive control forward primer
caggtgcaaatggccaactcg

SEQ ID NO: 14 - DNA, 19 bp, Artificial Sequence
  RGP group positive control reverse primer
cttgccatgttgggatgac

SEQ ID NO: 15 - DNA, 30 bp, Artificial Sequence
  Host1
gaatgatactgctggcagtatttcggttgg

SEQ ID NO: 16 - DNA, 31 bp, Artificial Sequence
  Host5
cagtcatgtagctatcgatgaaattccaacg

SEQ ID NO: 17 - DNA, 801 bp, Streptococcus thermophilus
  Positive control amplicon
caggtgcaaatggccaactcggaactgaacttcgtcacctacttgatgaacgtaacgaagagtatgtagcagtagatgtggcagaaatggacatcacagatgccgaaaaagtagatgaagtgtttgcggaagtaaaaccaaccttggtttatcactgtgctgcttacacagctgttgatgctgctgaagatgaaggcaaagagcttgactacgctattaacgtgactggtactgaaaatgtcgctaaggctgcagaaaaacatggtgcaacgcttgtttatatttcaacggactacgtttttaatggtgaaaaaccagtcggtcaagagtgggaagttgatgataaaccagatccacagacagagtatggtcgtacaaaacgtatgggtgaagagctagttgaaaaacatgtgactaactactacattatccgtacttcctgggtgttcggtaactatggtaaaaattttgtcttcactatgcaaaaccttgctaaaactcacaagacgctgacagtcgttaatgaccaacatggccgtccaacttggacacgtactttggcagagtttatgacttatttggctgaaaaccgtaaggaatatggttactatcacttgtcaaatgatgcaacagaagatacaacttggtatgactttgcggttgaaattctcaaagatactgatgttgaagtgaaacctgttgattcaagtcaattcccagctaaagctaaacgtcctcttaactcaacaatgagtttggctaaggctaaggcaacaggatttgtcatcccaacatggcaag